European Patent Application EP 4 772 634 A1, published July 8, 2026. Title: DOUBLE-STRANDED RNA TARGETING COAGULATION FACTOR XI. Applicant: Chia Tai Tianqing Pharmaceutical Group Co., Ltd. The sequence listing filed with the application follows.

SEQUENCE LISTING (84 sequences)

SEQ ID NO: 1 - RNA, 19 nt, synthetic construct
  source 1..19: mol_type = other RNA; note; note (original language) = sense strand
gatctccaactaaaatact

SEQ ID NO: 2 - RNA, 21 nt, synthetic construct
  source 1..21: mol_type = other RNA; note; note (original language) = antisense strand
agtattttagttggagatccg

SEQ ID NO: 3 - RNA, 19 nt, synthetic construct
  source 1..19: mol_type = other RNA; note; note (original language) = sense strand
ggatgattttcttatatca

SEQ ID NO: 4 - RNA, 21 nt, synthetic construct
  source 1..21: mol_type = other RNA; note; note (original language) = antisense strand
tgatataagaaaatcatcctg

SEQ ID NO: 5 - RNA, 19 nt, synthetic construct
  source 1..19: mol_type = other RNA; note; note (original language) = sense strand
ggtcttttcaggatgattt

SEQ ID NO: 6 - RNA, 21 nt, synthetic construct
  source 1..21: mol_type = other RNA; note; note (original language) = antisense strand
aaatcatcctgaaaagacctt

SEQ ID NO: 7 - RNA, 19 nt, synthetic construct
  source 1..19: mol_type = other RNA; note; note (original language) = sense strand
gtcttttcaggatgatttt

SEQ ID NO: 8 - RNA, 21 nt, synthetic construct
  source 1..21: mol_type = other RNA; note; note (original language) = antisense strand
aaaatcatcctgaaaagacct

SEQ ID NO: 9 - RNA, 19 nt, synthetic construct
  source 1..19: mol_type = other RNA; note; note (original language) = sense strand
cttttcaggatgattttct

SEQ ID NO: 10 - RNA, 21 nt, synthetic construct
  source 1..21: mol_type = other RNA; note; note (original language) = antisense strand
agaaaatcatcctgaaaagac

SEQ ID NO: 11 - RNA, 19 nt, synthetic construct
  source 1..19: mol_type = other RNA; note; note (original language) = sense strand
ttttcaggatgattttctt

SEQ ID NO: 12 - RNA, 21 nt, synthetic construct
  source 1..21: mol_type = other RNA; note; note (original language) = antisense strand
aagaaaatcatcctgaaaaga

SEQ ID NO: 13 - RNA, 19 nt, synthetic construct
  source 1..19: mol_type = other RNA; note; note (original language) = sense strand
tcaggatgattttcttata

SEQ ID NO: 14 - RNA, 21 nt, synthetic construct
  source 1..21: mol_type = other RNA; note; note (original language) = antisense strand
tataagaaaatcatcctgaaa

SEQ ID NO: 15 - RNA, 19 nt, synthetic construct
  source 1..19: mol_type = other RNA; note; note (original language) = sense strand
caggatgattttcttatat

SEQ ID NO: 16 - RNA, 21 nt, synthetic construct
  source 1..21: mol_type = other RNA; note; note (original language) = antisense strand
atataagaaaatcatcctgaa

SEQ ID NO: 17 - RNA, 19 nt, synthetic construct
  source 1..19: mol_type = other RNA; note; note (original language) = sense strand
aggatgattttcttatatc

SEQ ID NO: 18 - RNA, 21 nt, synthetic construct
  source 1..21: mol_type = other RNA; note; note (original language) = antisense strand
gatataagaaaatcatcctga

SEQ ID NO: 19 - RNA, 19 nt, synthetic construct
  source 1..19: mol_type = other RNA; note; note (original language) = sense strand
gatgattttcttatatcaa

SEQ ID NO: 20 - RNA, 21 nt, synthetic construct
  source 1..21: mol_type = other RNA; note; note (original language) = antisense strand
ttgatataagaaaatcatcct

SEQ ID NO: 21 - RNA, 19 nt, synthetic construct
  source 1..19: mol_type = other RNA; note; note (original language) = sense strand
atgattttcttatatcaag

SEQ ID NO: 22 - RNA, 21 nt, synthetic construct
  source 1..21: mol_type = other RNA; note; note (original language) = antisense strand
cttgatataagaaaatcatcc

SEQ ID NO: 23 - RNA, 19 nt, synthetic construct
  source 1..19: mol_type = other RNA; note; note (original language) = sense strand
tgattttcttatatcaagt

SEQ ID NO: 24 - RNA, 21 nt, synthetic construct
  source 1..21: mol_type = other RNA; note; note (original language) = antisense strand
acttgatataagaaaatcatc

SEQ ID NO: 25 - RNA, 19 nt, synthetic construct
  source 1..19: mol_type = other RNA; note; note (original language) = sense strand
cttatatcaagtggtacat

SEQ ID NO: 26 - RNA, 21 nt, synthetic construct
  source 1..21: mol_type = other RNA; note; note (original language) = antisense strand
atgtaccacttgatataagaa

SEQ ID NO: 27 - RNA, 19 nt, synthetic construct
  source 1..19: mol_type = other RNA; note; note (original language) = sense strand
aaacggatctccaactaaa

SEQ ID NO: 28 - RNA, 21 nt, synthetic construct
  source 1..21: mol_type = other RNA; note; note (original language) = antisense strand
tttagttggagatccgtttga

SEQ ID NO: 29 - RNA, 19 nt, synthetic construct
  source 1..19: mol_type = other RNA; note; note (original language) = sense strand
  modified_base 1..4: mod_base = OTHER; note; note (original language) = 2'-O-methyl modification
  modified_base 5: mod_base = OTHER; note; note (original language) = 2'-fluoro modification
  modified_base 6: mod_base = OTHER; note; note (original language) = 2'-O-methyl modification
  modified_base 7..9: mod_base = OTHER; note; note (original language) = 2'-fluoro modification
  modified_base 10..19: mod_base = OTHER; note; note (original language) = 2'-O-methyl modification
  modified_base 1^2: mod_base = OTHER; note; note (original language) = phosphorothioate linkage
  modified_base 2^3: mod_base = OTHER; note; note (original language) = phosphorothioate linkage
gatctccaactaaaatact

SEQ ID NO: 30 - RNA, 21 nt, synthetic construct
  source 1..21: mol_type = other RNA; note; note (original language) = antisense strand
  modified_base 1: mod_base = OTHER; note; note (original language) = 2'-O-methyl modification
  modified_base 2: mod_base = OTHER; note; note (original language) = 2'-fluoro modification
  modified_base 3..5: mod_base = OTHER; note; note (original language) = 2'-O-methyl modification
  modified_base 6: mod_base = OTHER; note; note (original language) = 2'-fluoro modification
  modified_base 7: mod_base = OTHER; note; note (original language) = 2'-O-methyl modification
  modified_base 8..9: mod_base = OTHER; note; note (original language) = 2'-fluoro modification
  modified_base 10..13: mod_base = OTHER; note; note (original language) = 2'-O-methyl modification
  modified_base 14: mod_base = OTHER; note; note (original language) = 2'-fluoro modification
  modified_base 15: mod_base = OTHER; note; note (original language) = 2'-O-methyl modification
  modified_base 16: mod_base = OTHER; note; note (original language) = 2'-fluoro modification
  modified_base 17..21: mod_base = OTHER; note; note (original language) = 2'-O-methyl modification
  modified_base 1^2: mod_base = OTHER; note; note (original language) = phosphorothioate linkage
  modified_base 2^3: mod_base = OTHER; note; note (original language) = phosphorothioate linkage
  modified_base 19^20: mod_base = OTHER; note; note (original language) = phosphorothioate linkage
  modified_base 20^21: mod_base = OTHER; note; note (original language) = phosphorothioate linkage
agtattttagttggagatccg

SEQ ID NO: 31 - RNA, 19 nt, synthetic construct
  source 1..19: mol_type = other RNA; note; note (original language) = sense strand
  modified_base 1..6: mod_base = OTHER; note; note (original language) = 2'-O-methyl modification
  modified_base 7..9: mod_base = OTHER; note; note (original language) = 2'-fluoro modification
  modified_base 10..19: mod_base = OTHER; note; note (original language) = 2'-O-methyl modification
  modified_base 1^2: mod_base = OTHER; note; note (original language) = phosphorothioate linkage
  modified_base 2^3: mod_base = OTHER; note; note (original language) = phosphorothioate linkage
gatctccaactaaaatact

SEQ ID NO: 32 - RNA, 21 nt, synthetic construct
  source 1..21: mol_type = other RNA; note; note (original language) = antisense strand
  modified_base 1: mod_base = OTHER; note; note (original language) = 2'-O-methyl modification
  modified_base 2: mod_base = OTHER; note; note (original language) = 2'-fluoro modification
  modified_base 3..5: mod_base = OTHER; note; note (original language) = 2'-O-methyl modification
  modified_base 6: mod_base = OTHER; note; note (original language) = 2'-fluoro modification
  modified_base 7..13: mod_base = OTHER; note; note (original language) = 2'-O-methyl modification
  modified_base 14: mod_base = OTHER; note; note (original language) = 2'-fluoro modification
  modified_base 15: mod_base = OTHER; note; note (original language) = 2'-O-methyl modification
  modified_base 16: mod_base = OTHER; note; note (original language) = 2'-fluoro modification
  modified_base 17..21: mod_base = OTHER; note; note (original language) = 2'-O-methyl modification
  modified_base 1^2: mod_base = OTHER; note; note (original language) = phosphorothioate linkage
  modified_base 2^3: mod_base = OTHER; note; note (original language) = phosphorothioate linkage
  modified_base 19^20: mod_base = OTHER; note; note (original language) = phosphorothioate linkage
  modified_base 20^21: mod_base = OTHER; note; note (original language) = phosphorothioate linkage
agtattttagttggagatccg

SEQ ID NO: 33 - RNA, 19 nt, synthetic construct
  source 1..19: mol_type = other RNA; note; note (original language) = sense strand
  modified_base 1..4: mod_base = OTHER; note; note (original language) = 2'-O-methyl modification
  modified_base 5: mod_base = OTHER; note; note (original language) = 2'-fluoro modification
  modified_base 6: mod_base = OTHER; note; note (original language) = 2'-O-methyl modification
  modified_base 7..9: mod_base = OTHER; note; note (original language) = 2'-fluoro modification
  modified_base 10..19: mod_base = OTHER; note; note (original language) = 2'-O-methyl modification
  modified_base 1^2: mod_base = OTHER; note; note (original language) = phosphorothioate linkage
  modified_base 2^3: mod_base = OTHER; note; note (original language) = phosphorothioate linkage
ggatgattttcttatatca

SEQ ID NO: 34 - RNA, 21 nt, synthetic construct
  source 1..21: mol_type = other RNA; note; note (original language) = antisense strand
  modified_base 1: mod_base = OTHER; note; note (original language) = 2'-O-methyl modification
  modified_base 2: mod_base = OTHER; note; note (original language) = 2'-fluoro modification
  modified_base 3..5: mod_base = OTHER; note; note (original language) = 2'-O-methyl modification
  modified_base 6: mod_base = OTHER; note; note (original language) = 2'-fluoro modification
  modified_base 7: mod_base = OTHER; note; note (original language) = 2'-O-methyl modification
  modified_base 8..9: mod_base = OTHER; note; note (original language) = 2'-fluoro modification
  modified_base 10..13: mod_base = OTHER; note; note (original language) = 2'-O-methyl modification
  modified_base 14: mod_base = OTHER; note; note (original language) = 2'-fluoro modification
  modified_base 15: mod_base = OTHER; note; note (original language) = 2'-O-methyl modification
  modified_base 16: mod_base = OTHER; note; note (original language) = 2'-fluoro modification
  modified_base 17..21: mod_base = OTHER; note; note (original language) = 2'-O-methyl modification
  modified_base 1^2: mod_base = OTHER; note; note (original language) = phosphorothioate linkage
  modified_base 2^3: mod_base = OTHER; note; note (original language) = phosphorothioate linkage
  modified_base 19^20: mod_base = OTHER; note; note (original language) = phosphorothioate linkage
  modified_base 20^21: mod_base = OTHER; note; note (original language) = phosphorothioate linkage
tgatataagaaaatcatcctg

SEQ ID NO: 35 - RNA, 19 nt, synthetic construct
  source 1..19: mol_type = other RNA; note; note (original language) = sense strand
  modified_base 1..6: mod_base = OTHER; note; note (original language) = 2'-O-methyl modification
  modified_base 7..9: mod_base = OTHER; note; note (original language) = 2'-fluoro modification
  modified_base 10..19: mod_base = OTHER; note; note (original language) = 2'-O-methyl modification
  modified_base 1^2: mod_base = OTHER; note; note (original language) = phosphorothioate linkage
  modified_base 2^3: mod_base = OTHER; note; note (original language) = phosphorothioate linkage
ggatgattttcttatatca

SEQ ID NO: 36 - RNA, 21 nt, synthetic construct
  source 1..21: mol_type = other RNA; note; note (original language) = antisense strand
  modified_base 1: mod_base = OTHER; note; note (original language) = 2'-O-methyl modification
  modified_base 2: mod_base = OTHER; note; note (original language) = 2'-fluoro modification
  modified_base 3..5: mod_base = OTHER; note; note (original language) = 2'-O-methyl modification
  modified_base 6: mod_base = OTHER; note; note (original language) = 2'-fluoro modification
  modified_base 7..13: mod_base = OTHER; note; note (original language) = 2'-O-methyl modification
  modified_base 14: mod_base = OTHER; note; note (original language) = 2'-fluoro modification
  modified_base 15: mod_base = OTHER; note; note (original language) = 2'-O-methyl modification
  modified_base 16: mod_base = OTHER; note; note (original language) = 2'-fluoro modification
  modified_base 17..21: mod_base = OTHER; note; note (original language) = 2'-O-methyl modification
  modified_base 1^2: mod_base = OTHER; note; note (original language) = phosphorothioate linkage
  modified_base 2^3: mod_base = OTHER; note; note (original language) = phosphorothioate linkage
  modified_base 19^20: mod_base = OTHER; note; note (original language) = phosphorothioate linkage
  modified_base 20^21: mod_base = OTHER; note; note (original language) = phosphorothioate linkage
tgatataagaaaatcatcctg

SEQ ID NO: 37 - RNA, 19 nt, synthetic construct
  source 1..19: mol_type = other RNA; note; note (original language) = sense strand
  modified_base 1..4: mod_base = OTHER; note; note (original language) = 2'-O-methyl modification
  modified_base 5: mod_base = OTHER; note; note (original language) = 2'-fluoro modification
  modified_base 6: mod_base = OTHER; note; note (original language) = 2'-O-methyl modification
  modified_base 7..9: mod_base = OTHER; note; note (original language) = 2'-fluoro modification
  modified_base 10..19: mod_base = OTHER; note; note (original language) = 2'-O-methyl modification
  modified_base 1^2: mod_base = OTHER; note; note (original language) = phosphorothioate linkage
  modified_base 2^3: mod_base = OTHER; note; note (original language) = phosphorothioate linkage
ggtcttttcaggatgattt

SEQ ID NO: 38 - RNA, 21 nt, synthetic construct
  source 1..21: mol_type = other RNA; note; note (original language) = antisense strand
  modified_base 1: mod_base = OTHER; note; note (original language) = 2'-O-methyl modification
  modified_base 2: mod_base = OTHER; note; note (original language) = 2'-fluoro modification
  modified_base 3..5: mod_base = OTHER; note; note (original language) = 2'-O-methyl modification
  modified_base 6: mod_base = OTHER; note; note (original language) = 2'-fluoro modification
  modified_base 7: mod_base = OTHER; note; note (original language) = 2'-O-methyl modification
  modified_base 8..9: mod_base = OTHER; note; note (original language) = 2'-fluoro modification
  modified_base 10..13: mod_base = OTHER; note; note (original language) = 2'-O-methyl modification
  modified_base 14: mod_base = OTHER; note; note (original language) = 2'-fluoro modification
  modified_base 15: mod_base = OTHER; note; note (original language) = 2'-O-methyl modification
  modified_base 16: mod_base = OTHER; note; note (original language) = 2'-fluoro modification
  modified_base 17..21: mod_base = OTHER; note; note (original language) = 2'-O-methyl modification
  modified_base 1^2: mod_base = OTHER; note; note (original language) = phosphorothioate linkage
  modified_base 2^3: mod_base = OTHER; note; note (original language) = phosphorothioate linkage
  modified_base 19^20: mod_base = OTHER; note; note (original language) = phosphorothioate linkage
  modified_base 20^21: mod_base = OTHER; note; note (original language) = phosphorothioate linkage
aaatcatcctgaaaagacctt

SEQ ID NO: 39 - RNA, 19 nt, synthetic construct
  source 1..19: mol_type = other RNA; note; note (original language) = sense strand
  modified_base 1..6: mod_base = OTHER; note; note (original language) = 2'-O-methyl modification
  modified_base 7..9: mod_base = OTHER; note; note (original language) = 2'-fluoro modification
  modified_base 10..19: mod_base = OTHER; note; note (original language) = 2'-O-methyl modification
  modified_base 1^2: mod_base = OTHER; note; note (original language) = phosphorothioate linkage
  modified_base 2^3: mod_base = OTHER; note; note (original language) = phosphorothioate linkage
ggtcttttcaggatgattt

SEQ ID NO: 40 - RNA, 21 nt, synthetic construct
  source 1..21: mol_type = other RNA; note; note (original language) = antisense strand
  modified_base 1: mod_base = OTHER; note; note (original language) = 2'-O-methyl modification
  modified_base 2: mod_base = OTHER; note; note (original language) = 2'-fluoro modification
  modified_base 3..5: mod_base = OTHER; note; note (original language) = 2'-O-methyl modification
  modified_base 6: mod_base = OTHER; note; note (original language) = 2'-fluoro modification
  modified_base 7..13: mod_base = OTHER; note; note (original language) = 2'-O-methyl modification
  modified_base 14: mod_base = OTHER; note; note (original language) = 2'-fluoro modification
  modified_base 15: mod_base = OTHER; note; note (original language) = 2'-O-methyl modification
  modified_base 16: mod_base = OTHER; note; note (original language) = 2'-fluoro modification
  modified_base 17..21: mod_base = OTHER; note; note (original language) = 2'-O-methyl modification
  modified_base 1^2: mod_base = OTHER; note; note (original language) = phosphorothioate linkage
  modified_base 2^3: mod_base = OTHER; note; note (original language) = phosphorothioate linkage
  modified_base 19^20: mod_base = OTHER; note; note (original language) = phosphorothioate linkage
  modified_base 20^21: mod_base = OTHER; note; note (original language) = phosphorothioate linkage
aaatcatcctgaaaagacctt

SEQ ID NO: 41 - RNA, 19 nt, synthetic construct
  source 1..19: mol_type = other RNA; note; note (original language) = sense strand
  modified_base 1..4: mod_base = OTHER; note; note (original language) = 2'-O-methyl modification
  modified_base 5: mod_base = OTHER; note; note (original language) = 2'-fluoro modification
  modified_base 6: mod_base = OTHER; note; note (original language) = 2'-O-methyl modification
  modified_base 7..9: mod_base = OTHER; note; note (original language) = 2'-fluoro modification
  modified_base 10..19: mod_base = OTHER; note; note (original language) = 2'-O-methyl modification
  modified_base 1^2: mod_base = OTHER; note; note (original language) = phosphorothioate linkage
  modified_base 2^3: mod_base = OTHER; note; note (original language) = phosphorothioate linkage
gtcttttcaggatgatttt

SEQ ID NO: 42 - RNA, 21 nt, synthetic construct
  source 1..21: mol_type = other RNA; note; note (original language) = antisense strand
  modified_base 1: mod_base = OTHER; note; note (original language) = 2'-O-methyl modification
  modified_base 2: mod_base = OTHER; note; note (original language) = 2'-fluoro modification
  modified_base 3..5: mod_base = OTHER; note; note (original language) = 2'-O-methyl modification
  modified_base 6: mod_base = OTHER; note; note (original language) = 2'-fluoro modification
  modified_base 7: mod_base = OTHER; note; note (original language) = 2'-O-methyl modification
  modified_base 8..9: mod_base = OTHER; note; note (original language) = 2'-fluoro modification
  modified_base 10..13: mod_base = OTHER; note; note (original language) = 2'-O-methyl modification
  modified_base 14: mod_base = OTHER; note; note (original language) = 2'-fluoro modification
  modified_base 15: mod_base = OTHER; note; note (original language) = 2'-O-methyl modification
  modified_base 16: mod_base = OTHER; note; note (original language) = 2'-fluoro modification
  modified_base 17..21: mod_base = OTHER; note; note (original language) = 2'-O-methyl modification
  modified_base 1^2: mod_base = OTHER; note; note (original language) = phosphorothioate linkage
  modified_base 2^3: mod_base = OTHER; note; note (original language) = phosphorothioate linkage
  modified_base 19^20: mod_base = OTHER; note; note (original language) = phosphorothioate linkage
  modified_base 20^21: mod_base = OTHER; note; note (original language) = phosphorothioate linkage
aaaatcatcctgaaaagacct

SEQ ID NO: 43 - RNA, 19 nt, synthetic construct
  source 1..19: mol_type = other RNA; note; note (original language) = sense strand
  modified_base 1..6: mod_base = OTHER; note; note (original language) = 2'-O-methyl modification
  modified_base 7..9: mod_base = OTHER; note; note (original language) = 2'-fluoro modification
  modified_base 10..19: mod_base = OTHER; note; note (original language) = 2'-O-methyl modification
  modified_base 1^2: mod_base = OTHER; note; note (original language) = phosphorothioate linkage
  modified_base 2^3: mod_base = OTHER; note; note (original language) = phosphorothioate linkage
gtcttttcaggatgatttt

SEQ ID NO: 44 - RNA, 21 nt, synthetic construct
  source 1..21: mol_type = other RNA; note; note (original language) = antisense strand
  modified_base 1: mod_base = OTHER; note; note (original language) = 2'-O-methyl modification
  modified_base 2: mod_base = OTHER; note; note (original language) = 2'-fluoro modification
  modified_base 3..5: mod_base = OTHER; note; note (original language) = 2'-O-methyl modification
  modified_base 6: mod_base = OTHER; note; note (original language) = 2'-fluoro modification
  modified_base 7..13: mod_base = OTHER; note; note (original language) = 2'-O-methyl modification
  modified_base 14: mod_base = OTHER; note; note (original language) = 2'-fluoro modification
  modified_base 15: mod_base = OTHER; note; note (original language) = 2'-O-methyl modification
  modified_base 16: mod_base = OTHER; note; note (original language) = 2'-fluoro modification
  modified_base 17..21: mod_base = OTHER; note; note (original language) = 2'-O-methyl modification
  modified_base 1^2: mod_base = OTHER; note; note (original language) = phosphorothioate linkage
  modified_base 2^3: mod_base = OTHER; note; note (original language) = phosphorothioate linkage
  modified_base 19^20: mod_base = OTHER; note; note (original language) = phosphorothioate linkage
  modified_base 20^21: mod_base = OTHER; note; note (original language) = phosphorothioate linkage
aaaatcatcctgaaaagacct

SEQ ID NO: 45 - RNA, 19 nt, synthetic construct
  source 1..19: mol_type = other RNA; note; note (original language) = sense strand
  modified_base 1..4: mod_base = OTHER; note; note (original language) = 2'-O-methyl modification
  modified_base 5: mod_base = OTHER; note; note (original language) = 2'-fluoro modification
  modified_base 6: mod_base = OTHER; note; note (original language) = 2'-O-methyl modification
  modified_base 7..9: mod_base = OTHER; note; note (original language) = 2'-fluoro modification
  modified_base 10..19: mod_base = OTHER; note; note (original language) = 2'-O-methyl modification
  modified_base 1^2: mod_base = OTHER; note; note (original language) = phosphorothioate linkage
  modified_base 2^3: mod_base = OTHER; note; note (original language) = phosphorothioate linkage
cttttcaggatgattttct

SEQ ID NO: 46 - RNA, 21 nt, synthetic construct
  source 1..21: mol_type = other RNA; note; note (original language) = antisense strand
  modified_base 1: mod_base = OTHER; note; note (original language) = 2'-O-methyl modification
  modified_base 2: mod_base = OTHER; note; note (original language) = 2'-fluoro modification
  modified_base 3..5: mod_base = OTHER; note; note (original language) = 2'-O-methyl modification
  modified_base 6: mod_base = OTHER; note; note (original language) = 2'-fluoro modification
  modified_base 7: mod_base = OTHER; note; note (original language) = 2'-O-methyl modification
  modified_base 8..9: mod_base = OTHER; note; note (original language) = 2'-fluoro modification
  modified_base 10..13: mod_base = OTHER; note; note (original language) = 2'-O-methyl modification
  modified_base 14: mod_base = OTHER; note; note (original language) = 2'-fluoro modification
  modified_base 15: mod_base = OTHER; note; note (original language) = 2'-O-methyl modification
  modified_base 16: mod_base = OTHER; note; note (original language) = 2'-fluoro modification
  modified_base 17..21: mod_base = OTHER; note; note (original language) = 2'-O-methyl modification
  modified_base 1^2: mod_base = OTHER; note; note (original language) = phosphorothioate linkage
  modified_base 2^3: mod_base = OTHER; note; note (original language) = phosphorothioate linkage
  modified_base 19^20: mod_base = OTHER; note; note (original language) = phosphorothioate linkage
  modified_base 20^21: mod_base = OTHER; note; note (original language) = phosphorothioate linkage
agaaaatcatcctgaaaagac

SEQ ID NO: 47 - RNA, 19 nt, synthetic construct
  source 1..19: mol_type = other RNA; note; note (original language) = sense strand
  modified_base 1..6: mod_base = OTHER; note; note (original language) = 2'-O-methyl modification
  modified_base 7..9: mod_base = OTHER; note; note (original language) = 2'-fluoro modification
  modified_base 10..19: mod_base = OTHER; note; note (original language) = 2'-O-methyl modification
  modified_base 1^2: mod_base = OTHER; note; note (original language) = phosphorothioate linkage
  modified_base 2^3: mod_base = OTHER; note; note (original language) = phosphorothioate linkage
cttttcaggatgattttct

SEQ ID NO: 48 - RNA, 21 nt, synthetic construct
  source 1..21: mol_type = other RNA; note; note (original language) = antisense strand
  modified_base 1: mod_base = OTHER; note; note (original language) = 2'-O-methyl modification
  modified_base 2: mod_base = OTHER; note; note (original language) = 2'-fluoro modification
  modified_base 3..5: mod_base = OTHER; note; note (original language) = 2'-O-methyl modification
  modified_base 6: mod_base = OTHER; note; note (original language) = 2'-fluoro modification
  modified_base 7..13: mod_base = OTHER; note; note (original language) = 2'-O-methyl modification
  modified_base 14: mod_base = OTHER; note; note (original language) = 2'-fluoro modification
  modified_base 15: mod_base = OTHER; note; note (original language) = 2'-O-methyl modification
  modified_base 16: mod_base = OTHER; note; note (original language) = 2'-fluoro modification
  modified_base 17..21: mod_base = OTHER; note; note (original language) = 2'-O-methyl modification
  modified_base 1^2: mod_base = OTHER; note; note (original language) = phosphorothioate linkage
  modified_base 2^3: mod_base = OTHER; note; note (original language) = phosphorothioate linkage
  modified_base 19^20: mod_base = OTHER; note; note (original language) = phosphorothioate linkage
  modified_base 20^21: mod_base = OTHER; note; note (original language) = phosphorothioate linkage
agaaaatcatcctgaaaagac

SEQ ID NO: 49 - RNA, 19 nt, synthetic construct
  source 1..19: mol_type = other RNA; note; note (original language) = sense strand
  modified_base 1..4: mod_base = OTHER; note; note (original language) = 2'-O-methyl modification
  modified_base 5: mod_base = OTHER; note; note (original language) = 2'-fluoro modification
  modified_base 6: mod_base = OTHER; note; note (original language) = 2'-O-methyl modification
  modified_base 7..9: mod_base = OTHER; note; note (original language) = 2'-fluoro modification
  modified_base 10..19: mod_base = OTHER; note; note (original language) = 2'-O-methyl modification
  modified_base 1^2: mod_base = OTHER; note; note (original language) = phosphorothioate linkage
  modified_base 2^3: mod_base = OTHER; note; note (original language) = phosphorothioate linkage
ttttcaggatgattttctt

SEQ ID NO: 50 - RNA, 21 nt, synthetic construct
  source 1..21: mol_type = other RNA; note; note (original language) = antisense strand
  modified_base 1: mod_base = OTHER; note; note (original language) = 2'-O-methyl modification
  modified_base 2: mod_base = OTHER; note; note (original language) = 2'-fluoro modification
  modified_base 3..5: mod_base = OTHER; note; note (original language) = 2'-O-methyl modification
  modified_base 6: mod_base = OTHER; note; note (original language) = 2'-fluoro modification
  modified_base 7: mod_base = OTHER; note; note (original language) = 2'-O-methyl modification
  modified_base 8..9: mod_base = OTHER; note; note (original language) = 2'-fluoro modification
  modified_base 10..13: mod_base = OTHER; note; note (original language) = 2'-O-methyl modification
  modified_base 14: mod_base = OTHER; note; note (original language) = 2'-fluoro modification
  modified_base 15: mod_base = OTHER; note; note (original language) = 2'-O-methyl modification
  modified_base 16: mod_base = OTHER; note; note (original language) = 2'-fluoro modification
  modified_base 17..21: mod_base = OTHER; note; note (original language) = 2'-O-methyl modification
  modified_base 1^2: mod_base = OTHER; note; note (original language) = phosphorothioate linkage
  modified_base 2^3: mod_base = OTHER; note; note (original language) = phosphorothioate linkage
  modified_base 19^20: mod_base = OTHER; note; note (original language) = phosphorothioate linkage
  modified_base 20^21: mod_base = OTHER; note; note (original language) = phosphorothioate linkage
aagaaaatcatcctgaaaaga

SEQ ID NO: 51 - RNA, 19 nt, synthetic construct
  source 1..19: mol_type = other RNA; note; note (original language) = sense strand
  modified_base 1..6: mod_base = OTHER; note; note (original language) = 2'-O-methyl modification
  modified_base 7..9: mod_base = OTHER; note; note (original language) = 2'-fluoro modification
  modified_base 10..19: mod_base = OTHER; note; note (original language) = 2'-O-methyl modification
  modified_base 1^2: mod_base = OTHER; note; note (original language) = phosphorothioate linkage
  modified_base 2^3: mod_base = OTHER; note; note (original language) = phosphorothioate linkage
ttttcaggatgattttctt

SEQ ID NO: 52 - RNA, 21 nt, synthetic construct
  source 1..21: mol_type = other RNA; note; note (original language) = antisense strand
  modified_base 1: mod_base = OTHER; note; note (original language) = 2'-O-methyl modification
  modified_base 2: mod_base = OTHER; note; note (original language) = 2'-fluoro modification
  modified_base 3..5: mod_base = OTHER; note; note (original language) = 2'-O-methyl modification
  modified_base 6: mod_base = OTHER; note; note (original language) = 2'-fluoro modification
  modified_base 7..13: mod_base = OTHER; note; note (original language) = 2'-O-methyl modification
  modified_base 14: mod_base = OTHER; note; note (original language) = 2'-fluoro modification
  modified_base 15: mod_base = OTHER; note; note (original language) = 2'-O-methyl modification
  modified_base 16: mod_base = OTHER; note; note (original language) = 2'-fluoro modification
  modified_base 17..21: mod_base = OTHER; note; note (original language) = 2'-O-methyl modification
  modified_base 1^2: mod_base = OTHER; note; note (original language) = phosphorothioate linkage
  modified_base 2^3: mod_base = OTHER; note; note (original language) = phosphorothioate linkage
  modified_base 19^20: mod_base = OTHER; note; note (original language) = phosphorothioate linkage
  modified_base 20^21: mod_base = OTHER; note; note (original language) = phosphorothioate linkage
aagaaaatcatcctgaaaaga

SEQ ID NO: 53 - RNA, 19 nt, synthetic construct
  source 1..19: mol_type = other RNA; note; note (original language) = sense strand
  modified_base 1..4: mod_base = OTHER; note; note (original language) = 2'-O-methyl modification
  modified_base 5: mod_base = OTHER; note; note (original language) = 2'-fluoro modification
  modified_base 6: mod_base = OTHER; note; note (original language) = 2'-O-methyl modification
  modified_base 7..9: mod_base = OTHER; note; note (original language) = 2'-fluoro modification
  modified_base 10..19: mod_base = OTHER; note; note (original language) = 2'-O-methyl modification
  modified_base 1^2: mod_base = OTHER; note; note (original language) = phosphorothioate linkage
  modified_base 2^3: mod_base = OTHER; note; note (original language) = phosphorothioate linkage
tcaggatgattttcttata

SEQ ID NO: 54 - RNA, 21 nt, synthetic construct
  source 1..21: mol_type = other RNA; note; note (original language) = antisense strand
  modified_base 1: mod_base = OTHER; note; note (original language) = 2'-O-methyl modification
  modified_base 2: mod_base = OTHER; note; note (original language) = 2'-fluoro modification
  modified_base 3..5: mod_base = OTHER; note; note (original language) = 2'-O-methyl modification
  modified_base 6: mod_base = OTHER; note; note (original language) = 2'-fluoro modification
  modified_base 7: mod_base = OTHER; note; note (original language) = 2'-O-methyl modification
  modified_base 8..9: mod_base = OTHER; note; note (original language) = 2'-fluoro modification
  modified_base 10..13: mod_base = OTHER; note; note (original language) = 2'-O-methyl modification
  modified_base 14: mod_base = OTHER; note; note (original language) = 2'-fluoro modification
  modified_base 15: mod_base = OTHER; note; note (original language) = 2'-O-methyl modification
  modified_base 16: mod_base = OTHER; note; note (original language) = 2'-fluoro modification
  modified_base 17..21: mod_base = OTHER; note; note (original language) = 2'-O-methyl modification
  modified_base 1^2: mod_base = OTHER; note; note (original language) = phosphorothioate linkage
  modified_base 2^3: mod_base = OTHER; note; note (original language) = phosphorothioate linkage
  modified_base 19^20: mod_base = OTHER; note; note (original language) = phosphorothioate linkage
  modified_base 20^21: mod_base = OTHER; note; note (original language) = phosphorothioate linkage
tataagaaaatcatcctgaaa

SEQ ID NO: 55 - RNA, 19 nt, synthetic construct
  source 1..19: mol_type = other RNA; note; note (original language) = sense strand
  modified_base 1..6: mod_base = OTHER; note; note (original language) = 2'-O-methyl modification
  modified_base 7..9: mod_base = OTHER; note; note (original language) = 2'-fluoro modification
  modified_base 10..19: mod_base = OTHER; note; note (original language) = 2'-O-methyl modification
  modified_base 1^2: mod_base = OTHER; note; note (original language) = phosphorothioate linkage
  modified_base 2^3: mod_base = OTHER; note; note (original language) = phosphorothioate linkage
tcaggatgattttcttata

SEQ ID NO: 56 - RNA, 21 nt, synthetic construct
  source 1..21: mol_type = other RNA; note; note (original language) = antisense strand
  modified_base 1: mod_base = OTHER; note; note (original language) = 2'-O-methyl modification
  modified_base 2: mod_base = OTHER; note; note (original language) = 2'-fluoro modification
  modified_base 3..5: mod_base = OTHER; note; note (original language) = 2'-O-methyl modification
  modified_base 6: mod_base = OTHER; note; note (original language) = 2'-fluoro modification
  modified_base 7..13: mod_base = OTHER; note; note (original language) = 2'-O-methyl modification
  modified_base 14: mod_base = OTHER; note; note (original language) = 2'-fluoro modification
  modified_base 15: mod_base = OTHER; note; note (original language) = 2'-O-methyl modification
  modified_base 16: mod_base = OTHER; note; note (original language) = 2'-fluoro modification
  modified_base 17..21: mod_base = OTHER; note; note (original language) = 2'-O-methyl modification
  modified_base 1^2: mod_base = OTHER; note; note (original language) = phosphorothioate linkage
  modified_base 2^3: mod_base = OTHER; note; note (original language) = phosphorothioate linkage
  modified_base 19^20: mod_base = OTHER; note; note (original language) = phosphorothioate linkage
  modified_base 20^21: mod_base = OTHER; note; note (original language) = phosphorothioate linkage
tataagaaaatcatcctgaaa

SEQ ID NO: 57 - RNA, 19 nt, synthetic construct
  source 1..19: mol_type = other RNA; note; note (original language) = sense strand
  modified_base 1..4: mod_base = OTHER; note; note (original language) = 2'-O-methyl modification
  modified_base 5: mod_base = OTHER; note; note (original language) = 2'-fluoro modification
  modified_base 6: mod_base = OTHER; note; note (original language) = 2'-O-methyl modification
  modified_base 7..9: mod_base = OTHER; note; note (original language) = 2'-fluoro modification
  modified_base 10..19: mod_base = OTHER; note; note (original language) = 2'-O-methyl modification
  modified_base 1^2: mod_base = OTHER; note; note (original language) = phosphorothioate linkage
  modified_base 2^3: mod_base = OTHER; note; note (original language) = phosphorothioate linkage
caggatgattttcttatat

SEQ ID NO: 58 - RNA, 21 nt, synthetic construct
  source 1..21: mol_type = other RNA; note; note (original language) = antisense strand
  modified_base 1: mod_base = OTHER; note; note (original language) = 2'-O-methyl modification
  modified_base 2: mod_base = OTHER; note; note (original language) = 2'-fluoro modification
  modified_base 3..5: mod_base = OTHER; note; note (original language) = 2'-O-methyl modification
  modified_base 6: mod_base = OTHER; note; note (original language) = 2'-fluoro modification
  modified_base 7: mod_base = OTHER; note; note (original language) = 2'-O-methyl modification
  modified_base 8..9: mod_base = OTHER; note; note (original language) = 2'-fluoro modification
  modified_base 10..13: mod_base = OTHER; note; note (original language) = 2'-O-methyl modification
  modified_base 14: mod_base = OTHER; note; note (original language) = 2'-fluoro modification
  modified_base 15: mod_base = OTHER; note; note (original language) = 2'-O-methyl modification
  modified_base 16: mod_base = OTHER; note; note (original language) = 2'-fluoro modification
  modified_base 17..21: mod_base = OTHER; note; note (original language) = 2'-O-methyl modification
  modified_base 1^2: mod_base = OTHER; note; note (original language) = phosphorothioate linkage
  modified_base 2^3: mod_base = OTHER; note; note (original language) = phosphorothioate linkage
  modified_base 19^20: mod_base = OTHER; note; note (original language) = phosphorothioate linkage
  modified_base 20^21: mod_base = OTHER; note; note (original language) = phosphorothioate linkage
atataagaaaatcatcctgaa

SEQ ID NO: 59 - RNA, 19 nt, synthetic construct
  source 1..19: mol_type = other RNA; note; note (original language) = sense strand
  modified_base 1..6: mod_base = OTHER; note; note (original language) = 2'-O-methyl modification
  modified_base 7..9: mod_base = OTHER; note; note (original language) = 2'-fluoro modification
  modified_base 10..19: mod_base = OTHER; note; note (original language) = 2'-O-methyl modification
  modified_base 1^2: mod_base = OTHER; note; note (original language) = phosphorothioate linkage
  modified_base 2^3: mod_base = OTHER; note; note (original language) = phosphorothioate linkage
caggatgattttcttatat

SEQ ID NO: 60 - RNA, 21 nt, synthetic construct
  source 1..21: mol_type = other RNA; note; note (original language) = antisense strand
  modified_base 1: mod_base = OTHER; note; note (original language) = 2'-O-methyl modification
  modified_base 2: mod_base = OTHER; note; note (original language) = 2'-fluoro modification
  modified_base 3..5: mod_base = OTHER; note; note (original language) = 2'-O-methyl modification
  modified_base 6: mod_base = OTHER; note; note (original language) = 2'-fluoro modification
  modified_base 7..13: mod_base = OTHER; note; note (original language) = 2'-O-methyl modification
  modified_base 14: mod_base = OTHER; note; note (original language) = 2'-fluoro modification
  modified_base 15: mod_base = OTHER; note; note (original language) = 2'-O-methyl modification
  modified_base 16: mod_base = OTHER; note; note (original language) = 2'-fluoro modification
  modified_base 17..21: mod_base = OTHER; note; note (original language) = 2'-O-methyl modification
  modified_base 1^2: mod_base = OTHER; note; note (original language) = phosphorothioate linkage
  modified_base 2^3: mod_base = OTHER; note; note (original language) = phosphorothioate linkage
  modified_base 19^20: mod_base = OTHER; note; note (original language) = phosphorothioate linkage
  modified_base 20^21: mod_base = OTHER; note; note (original language) = phosphorothioate linkage
atataagaaaatcatcctgaa

SEQ ID NO: 61 - RNA, 19 nt, synthetic construct
  source 1..19: mol_type = other RNA; note; note (original language) = sense strand
  modified_base 1..4: mod_base = OTHER; note; note (original language) = 2'-O-methyl modification
  modified_base 5: mod_base = OTHER; note; note (original language) = 2'-fluoro modification
  modified_base 6: mod_base = OTHER; note; note (original language) = 2'-O-methyl modification
  modified_base 7..9: mod_base = OTHER; note; note (original language) = 2'-fluoro modification
  modified_base 10..19: mod_base = OTHER; note; note (original language) = 2'-O-methyl modification
  modified_base 1^2: mod_base = OTHER; note; note (original language) = phosphorothioate linkage
  modified_base 2^3: mod_base = OTHER; note; note (original language) = phosphorothioate linkage
aggatgattttcttatatc

SEQ ID NO: 62 - RNA, 21 nt, synthetic construct
  source 1..21: mol_type = other RNA; note; note (original language) = antisense strand
  modified_base 1: mod_base = OTHER; note; note (original language) = 2'-O-methyl modification
  modified_base 2: mod_base = OTHER; note; note (original language) = 2'-fluoro modification
  modified_base 3..5: mod_base = OTHER; note; note (original language) = 2'-O-methyl modification
  modified_base 6: mod_base = OTHER; note; note (original language) = 2'-fluoro modification
  modified_base 7: mod_base = OTHER; note; note (original language) = 2'-O-methyl modification
  modified_base 8..9: mod_base = OTHER; note; note (original language) = 2'-fluoro modification
  modified_base 10..13: mod_base = OTHER; note; note (original language) = 2'-O-methyl modification
  modified_base 14: mod_base = OTHER; note; note (original language) = 2'-fluoro modification
  modified_base 15: mod_base = OTHER; note; note (original language) = 2'-O-methyl modification
  modified_base 16: mod_base = OTHER; note; note (original language) = 2'-fluoro modification
  modified_base 17..21: mod_base = OTHER; note; note (original language) = 2'-O-methyl modification
  modified_base 1^2: mod_base = OTHER; note; note (original language) = phosphorothioate linkage
  modified_base 2^3: mod_base = OTHER; note; note (original language) = phosphorothioate linkage
  modified_base 19^20: mod_base = OTHER; note; note (original language) = phosphorothioate linkage
  modified_base 20^21: mod_base = OTHER; note; note (original language) = phosphorothioate linkage
gatataagaaaatcatcctga

SEQ ID NO: 63 - RNA, 19 nt, synthetic construct
  source 1..19: mol_type = other RNA; note; note (original language) = sense strand
  modified_base 1..6: mod_base = OTHER; note; note (original language) = 2'-O-methyl modification
  modified_base 7..9: mod_base = OTHER; note; note (original language) = 2'-fluoro modification
  modified_base 10..19: mod_base = OTHER; note; note (original language) = 2'-O-methyl modification
  modified_base 1^2: mod_base = OTHER; note; note (original language) = phosphorothioate linkage
  modified_base 2^3: mod_base = OTHER; note; note (original language) = phosphorothioate linkage
aggatgattttcttatatc

SEQ ID NO: 64 - RNA, 21 nt, synthetic construct
  source 1..21: mol_type = other RNA; note; note (original language) = antisense strand
  modified_base 1: mod_base = OTHER; note; note (original language) = 2'-O-methyl modification
  modified_base 2: mod_base = OTHER; note; note (original language) = 2'-fluoro modification
  modified_base 3..5: mod_base = OTHER; note; note (original language) = 2'-O-methyl modification
  modified_base 6: mod_base = OTHER; note; note (original language) = 2'-fluoro modification
  modified_base 7..13: mod_base = OTHER; note; note (original language) = 2'-O-methyl modification
  modified_base 14: mod_base = OTHER; note; note (original language) = 2'-fluoro modification
  modified_base 15: mod_base = OTHER; note; note (original language) = 2'-O-methyl modification
  modified_base 16: mod_base = OTHER; note; note (original language) = 2'-fluoro modification
  modified_base 17..21: mod_base = OTHER; note; note (original language) = 2'-O-methyl modification
  modified_base 1^2: mod_base = OTHER; note; note (original language) = phosphorothioate linkage
  modified_base 2^3: mod_base = OTHER; note; note (original language) = phosphorothioate linkage
  modified_base 19^20: mod_base = OTHER; note; note (original language) = phosphorothioate linkage
  modified_base 20^21: mod_base = OTHER; note; note (original language) = phosphorothioate linkage
gatataagaaaatcatcctga

SEQ ID NO: 65 - RNA, 19 nt, synthetic construct
  source 1..19: mol_type = other RNA; note; note (original language) = sense strand
  modified_base 1..4: mod_base = OTHER; note; note (original language) = 2'-O-methyl modification
  modified_base 5: mod_base = OTHER; note; note (original language) = 2'-fluoro modification
  modified_base 6: mod_base = OTHER; note; note (original language) = 2'-O-methyl modification
  modified_base 7..9: mod_base = OTHER; note; note (original language) = 2'-fluoro modification
  modified_base 10..19: mod_base = OTHER; note; note (original language) = 2'-O-methyl modification
  modified_base 1^2: mod_base = OTHER; note; note (original language) = phosphorothioate linkage
  modified_base 2^3: mod_base = OTHER; note; note (original language) = phosphorothioate linkage
gatgattttcttatatcaa

SEQ ID NO: 66 - RNA, 21 nt, synthetic construct
  source 1..21: mol_type = other RNA; note; note (original language) = antisense strand
  modified_base 1: mod_base = OTHER; note; note (original language) = 2'-O-methyl modification
  modified_base 2: mod_base = OTHER; note; note (original language) = 2'-fluoro modification
  modified_base 3..5: mod_base = OTHER; note; note (original language) = 2'-O-methyl modification
  modified_base 6: mod_base = OTHER; note; note (original language) = 2'-fluoro modification
  modified_base 7: mod_base = OTHER; note; note (original language) = 2'-O-methyl modification
  modified_base 8..9: mod_base = OTHER; note; note (original language) = 2'-fluoro modification
  modified_base 10..13: mod_base = OTHER; note; note (original language) = 2'-O-methyl modification
  modified_base 14: mod_base = OTHER; note; note (original language) = 2'-fluoro modification
  modified_base 15: mod_base = OTHER; note; note (original language) = 2'-O-methyl modification
  modified_base 16: mod_base = OTHER; note; note (original language) = 2'-fluoro modification
  modified_base 17..21: mod_base = OTHER; note; note (original language) = 2'-O-methyl modification
  modified_base 1^2: mod_base = OTHER; note; note (original language) = phosphorothioate linkage
  modified_base 2^3: mod_base = OTHER; note; note (original language) = phosphorothioate linkage
  modified_base 19^20: mod_base = OTHER; note; note (original language) = phosphorothioate linkage
  modified_base 20^21: mod_base = OTHER; note; note (original language) = phosphorothioate linkage
ttgatataagaaaatcatcct

SEQ ID NO: 67 - RNA, 19 nt, synthetic construct
  source 1..19: mol_type = other RNA; note; note (original language) = sense strand
  modified_base 1..6: mod_base = OTHER; note; note (original language) = 2'-O-methyl modification
  modified_base 7..9: mod_base = OTHER; note; note (original language) = 2'-fluoro modification
  modified_base 10..19: mod_base = OTHER; note; note (original language) = 2'-O-methyl modification
  modified_base 1^2: mod_base = OTHER; note; note (original language) = phosphorothioate linkage
  modified_base 2^3: mod_base = OTHER; note; note (original language) = phosphorothioate linkage
gatgattttcttatatcaa

SEQ ID NO: 68 - RNA, 21 nt, synthetic construct
  source 1..21: mol_type = other RNA; note; note (original language) = antisense strand
  modified_base 1: mod_base = OTHER; note; note (original language) = 2'-O-methyl modification
  modified_base 2: mod_base = OTHER; note; note (original language) = 2'-fluoro modification
  modified_base 3..5: mod_base = OTHER; note; note (original language) = 2'-O-methyl modification
  modified_base 6: mod_base = OTHER; note; note (original language) = 2'-fluoro modification
  modified_base 7..13: mod_base = OTHER; note; note (original language) = 2'-O-methyl modification
  modified_base 14: mod_base = OTHER; note; note (original language) = 2'-fluoro modification
  modified_base 15: mod_base = OTHER; note; note (original language) = 2'-O-methyl modification
  modified_base 16: mod_base = OTHER; note; note (original language) = 2'-fluoro modification
  modified_base 17..21: mod_base = OTHER; note; note (original language) = 2'-O-methyl modification
  modified_base 1^2: mod_base = OTHER; note; note (original language) = phosphorothioate linkage
  modified_base 2^3: mod_base = OTHER; note; note (original language) = phosphorothioate linkage
  modified_base 19^20: mod_base = OTHER; note; note (original language) = phosphorothioate linkage
  modified_base 20^21: mod_base = OTHER; note; note (original language) = phosphorothioate linkage
ttgatataagaaaatcatcct

SEQ ID NO: 69 - RNA, 19 nt, synthetic construct
  source 1..19: mol_type = other RNA; note; note (original language) = sense strand
  modified_base 1..4: mod_base = OTHER; note; note (original language) = 2'-O-methyl modification
  modified_base 5: mod_base = OTHER; note; note (original language) = 2'-fluoro modification
  modified_base 6: mod_base = OTHER; note; note (original language) = 2'-O-methyl modification
  modified_base 7..9: mod_base = OTHER; note; note (original language) = 2'-fluoro modification
  modified_base 10..19: mod_base = OTHER; note; note (original language) = 2'-O-methyl modification
  modified_base 1^2: mod_base = OTHER; note; note (original language) = phosphorothioate linkage
  modified_base 2^3: mod_base = OTHER; note; note (original language) = phosphorothioate linkage
atgattttcttatatcaag

SEQ ID NO: 70 - RNA, 21 nt, synthetic construct
  source 1..21: mol_type = other RNA; note; note (original language) = antisense strand
  modified_base 1: mod_base = OTHER; note; note (original language) = 2'-O-methyl modification
  modified_base 2: mod_base = OTHER; note; note (original language) = 2'-fluoro modification
  modified_base 3..5: mod_base = OTHER; note; note (original language) = 2'-O-methyl modification
  modified_base 6: mod_base = OTHER; note; note (original language) = 2'-fluoro modification
  modified_base 7: mod_base = OTHER; note; note (original language) = 2'-O-methyl modification
  modified_base 8..9: mod_base = OTHER; note; note (original language) = 2'-fluoro modification
  modified_base 10..13: mod_base = OTHER; note; note (original language) = 2'-O-methyl modification
  modified_base 14: mod_base = OTHER; note; note (original language) = 2'-fluoro modification
  modified_base 15: mod_base = OTHER; note; note (original language) = 2'-O-methyl modification
  modified_base 16: mod_base = OTHER; note; note (original language) = 2'-fluoro modification
  modified_base 17..21: mod_base = OTHER; note; note (original language) = 2'-O-methyl modification
  modified_base 1^2: mod_base = OTHER; note; note (original language) = phosphorothioate linkage
  modified_base 2^3: mod_base = OTHER; note; note (original language) = phosphorothioate linkage
  modified_base 19^20: mod_base = OTHER; note; note (original language) = phosphorothioate linkage
  modified_base 20^21: mod_base = OTHER; note; note (original language) = phosphorothioate linkage
cttgatataagaaaatcatcc

SEQ ID NO: 71 - RNA, 19 nt, synthetic construct
  source 1..19: mol_type = other RNA; note; note (original language) = sense strand
  modified_base 1..6: mod_base = OTHER; note; note (original language) = 2'-O-methyl modification
  modified_base 7..9: mod_base = OTHER; note; note (original language) = 2'-fluoro modification
  modified_base 10..19: mod_base = OTHER; note; note (original language) = 2'-O-methyl modification
  modified_base 1^2: mod_base = OTHER; note; note (original language) = phosphorothioate linkage
  modified_base 2^3: mod_base = OTHER; note; note (original language) = phosphorothioate linkage
atgattttcttatatcaag

SEQ ID NO: 72 - RNA, 21 nt, synthetic construct
  source 1..21: mol_type = other RNA; note; note (original language) = antisense strand
  modified_base 1: mod_base = OTHER; note; note (original language) = 2'-O-methyl modification
  modified_base 2: mod_base = OTHER; note; note (original language) = 2'-fluoro modification
  modified_base 3..5: mod_base = OTHER; note; note (original language) = 2'-O-methyl modification
  modified_base 6: mod_base = OTHER; note; note (original language) = 2'-fluoro modification
  modified_base 7..13: mod_base = OTHER; note; note (original language) = 2'-O-methyl modification
  modified_base 14: mod_base = OTHER; note; note (original language) = 2'-fluoro modification
  modified_base 15: mod_base = OTHER; note; note (original language) = 2'-O-methyl modification
  modified_base 16: mod_base = OTHER; note; note (original language) = 2'-fluoro modification
  modified_base 17..21: mod_base = OTHER; note; note (original language) = 2'-O-methyl modification
  modified_base 1^2: mod_base = OTHER; note; note (original language) = phosphorothioate linkage
  modified_base 2^3: mod_base = OTHER; note; note (original language) = phosphorothioate linkage
  modified_base 19^20: mod_base = OTHER; note; note (original language) = phosphorothioate linkage
  modified_base 20^21: mod_base = OTHER; note; note (original language) = phosphorothioate linkage
cttgatataagaaaatcatcc

SEQ ID NO: 73 - RNA, 19 nt, synthetic construct
  source 1..19: mol_type = other RNA; note; note (original language) = sense strand
  modified_base 1..4: mod_base = OTHER; note; note (original language) = 2'-O-methyl modification
  modified_base 5: mod_base = OTHER; note; note (original language) = 2'-fluoro modification
  modified_base 6: mod_base = OTHER; note; note (original language) = 2'-O-methyl modification
  modified_base 7..9: mod_base = OTHER; note; note (original language) = 2'-fluoro modification
  modified_base 10..19: mod_base = OTHER; note; note (original language) = 2'-O-methyl modification
  modified_base 1^2: mod_base = OTHER; note; note (original language) = phosphorothioate linkage
  modified_base 2^3: mod_base = OTHER; note; note (original language) = phosphorothioate linkage
tgattttcttatatcaagt

SEQ ID NO: 74 - RNA, 21 nt, synthetic construct
  source 1..21: mol_type = other RNA; note; note (original language) = antisense strand
  modified_base 1: mod_base = OTHER; note; note (original language) = 2'-O-methyl modification
  modified_base 2: mod_base = OTHER; note; note (original language) = 2'-fluoro modification
  modified_base 3..5: mod_base = OTHER; note; note (original language) = 2'-O-methyl modification
  modified_base 6: mod_base = OTHER; note; note (original language) = 2'-fluoro modification
  modified_base 7: mod_base = OTHER; note; note (original language) = 2'-O-methyl modification
  modified_base 8..9: mod_base = OTHER; note; note (original language) = 2'-fluoro modification
  modified_base 10..13: mod_base = OTHER; note; note (original language) = 2'-O-methyl modification
  modified_base 14: mod_base = OTHER; note; note (original language) = 2'-fluoro modification
  modified_base 15: mod_base = OTHER; note; note (original language) = 2'-O-methyl modification
  modified_base 16: mod_base = OTHER; note; note (original language) = 2'-fluoro modification
  modified_base 17..21: mod_base = OTHER; note; note (original language) = 2'-O-methyl modification
  modified_base 1^2: mod_base = OTHER; note; note (original language) = phosphorothioate linkage
  modified_base 2^3: mod_base = OTHER; note; note (original language) = phosphorothioate linkage
  modified_base 19^20: mod_base = OTHER; note; note (original language) = phosphorothioate linkage
  modified_base 20^21: mod_base = OTHER; note; note (original language) = phosphorothioate linkage
acttgatataagaaaatcatc

SEQ ID NO: 75 - RNA, 19 nt, synthetic construct
  source 1..19: mol_type = other RNA; note; note (original language) = sense strand
  modified_base 1..6: mod_base = OTHER; note; note (original language) = 2'-O-methyl modification
  modified_base 7..9: mod_base = OTHER; note; note (original language) = 2'-fluoro modification
  modified_base 10..19: mod_base = OTHER; note; note (original language) = 2'-O-methyl modification
  modified_base 1^2: mod_base = OTHER; note; note (original language) = phosphorothioate linkage
  modified_base 2^3: mod_base = OTHER; note; note (original language) = phosphorothioate linkage
tgattttcttatatcaagt

SEQ ID NO: 76 - RNA, 21 nt, synthetic construct
  source 1..21: mol_type = other RNA; note; note (original language) = antisense strand
  modified_base 1: mod_base = OTHER; note; note (original language) = 2'-O-methyl modification
  modified_base 2: mod_base = OTHER; note; note (original language) = 2'-fluoro modification
  modified_base 3..5: mod_base = OTHER; note; note (original language) = 2'-O-methyl modification
  modified_base 6: mod_base = OTHER; note; note (original language) = 2'-fluoro modification
  modified_base 7..13: mod_base = OTHER; note; note (original language) = 2'-O-methyl modification
  modified_base 14: mod_base = OTHER; note; note (original language) = 2'-fluoro modification
  modified_base 15: mod_base = OTHER; note; note (original language) = 2'-O-methyl modification
  modified_base 16: mod_base = OTHER; note; note (original language) = 2'-fluoro modification
  modified_base 17..21: mod_base = OTHER; note; note (original language) = 2'-O-methyl modification
  modified_base 1^2: mod_base = OTHER; note; note (original language) = phosphorothioate linkage
  modified_base 2^3: mod_base = OTHER; note; note (original language) = phosphorothioate linkage
  modified_base 19^20: mod_base = OTHER; note; note (original language) = phosphorothioate linkage
  modified_base 20^21: mod_base = OTHER; note; note (original language) = phosphorothioate linkage
acttgatataagaaaatcatc

SEQ ID NO: 77 - RNA, 19 nt, synthetic construct
  source 1..19: mol_type = other RNA; note; note (original language) = sense strand
  modified_base 1..4: mod_base = OTHER; note; note (original language) = 2'-O-methyl modification
  modified_base 5: mod_base = OTHER; note; note (original language) = 2'-fluoro modification
  modified_base 6: mod_base = OTHER; note; note (original language) = 2'-O-methyl modification
  modified_base 7..9: mod_base = OTHER; note; note (original language) = 2'-fluoro modification
  modified_base 10..19: mod_base = OTHER; note; note (original language) = 2'-O-methyl modification
  modified_base 1^2: mod_base = OTHER; note; note (original language) = phosphorothioate linkage
  modified_base 2^3: mod_base = OTHER; note; note (original language) = phosphorothioate linkage
cttatatcaagtggtacat

SEQ ID NO: 78 - RNA, 21 nt, synthetic construct
  source 1..21: mol_type = other RNA; note; note (original language) = antisense strand
  modified_base 1: mod_base = OTHER; note; note (original language) = 2'-O-methyl modification
  modified_base 2: mod_base = OTHER; note; note (original language) = 2'-fluoro modification
  modified_base 3..5: mod_base = OTHER; note; note (original language) = 2'-O-methyl modification
  modified_base 6: mod_base = OTHER; note; note (original language) = 2'-fluoro modification
  modified_base 7: mod_base = OTHER; note; note (original language) = 2'-O-methyl modification
  modified_base 8..9: mod_base = OTHER; note; note (original language) = 2'-fluoro modification
  modified_base 10..13: mod_base = OTHER; note; note (original language) = 2'-O-methyl modification
  modified_base 14: mod_base = OTHER; note; note (original language) = 2'-fluoro modification
  modified_base 15: mod_base = OTHER; note; note (original language) = 2'-O-methyl modification
  modified_base 16: mod_base = OTHER; note; note (original language) = 2'-fluoro modification
  modified_base 17..21: mod_base = OTHER; note; note (original language) = 2'-O-methyl modification
  modified_base 1^2: mod_base = OTHER; note; note (original language) = phosphorothioate linkage
  modified_base 2^3: mod_base = OTHER; note; note (original language) = phosphorothioate linkage
  modified_base 19^20: mod_base = OTHER; note; note (original language) = phosphorothioate linkage
  modified_base 20^21: mod_base = OTHER; note; note (original language) = phosphorothioate linkage
atgtaccacttgatataagaa

SEQ ID NO: 79 - RNA, 19 nt, synthetic construct
  source 1..19: mol_type = other RNA; note; note (original language) = sense strand
  modified_base 1..6: mod_base = OTHER; note; note (original language) = 2'-O-methyl modification
  modified_base 7..9: mod_base = OTHER; note; note (original language) = 2'-fluoro modification
  modified_base 10..19: mod_base = OTHER; note; note (original language) = 2'-O-methyl modification
  modified_base 1^2: mod_base = OTHER; note; note (original language) = phosphorothioate linkage
  modified_base 2^3: mod_base = OTHER; note; note (original language) = phosphorothioate linkage
cttatatcaagtggtacat

SEQ ID NO: 80 - RNA, 21 nt, synthetic construct
  source 1..21: mol_type = other RNA; note; note (original language) = antisense strand
  modified_base 1: mod_base = OTHER; note; note (original language) = 2'-O-methyl modification
  modified_base 2: mod_base = OTHER; note; note (original language) = 2'-fluoro modification
  modified_base 3..5: mod_base = OTHER; note; note (original language) = 2'-O-methyl modification
  modified_base 6: mod_base = OTHER; note; note (original language) = 2'-fluoro modification
  modified_base 7..13: mod_base = OTHER; note; note (original language) = 2'-O-methyl modification
  modified_base 14: mod_base = OTHER; note; note (original language) = 2'-fluoro modification
  modified_base 15: mod_base = OTHER; note; note (original language) = 2'-O-methyl modification
  modified_base 16: mod_base = OTHER; note; note (original language) = 2'-fluoro modification
  modified_base 17..21: mod_base = OTHER; note; note (original language) = 2'-O-methyl modification
  modified_base 1^2: mod_base = OTHER; note; note (original language) = phosphorothioate linkage
  modified_base 2^3: mod_base = OTHER; note; note (original language) = phosphorothioate linkage
  modified_base 19^20: mod_base = OTHER; note; note (original language) = phosphorothioate linkage
  modified_base 20^21: mod_base = OTHER; note; note (original language) = phosphorothioate linkage
atgtaccacttgatataagaa

SEQ ID NO: 81 - RNA, 19 nt, synthetic construct
  source 1..19: mol_type = other RNA; note; note (original language) = sense strand
  modified_base 1..4: mod_base = OTHER; note; note (original language) = 2'-O-methyl modification
  modified_base 5: mod_base = OTHER; note; note (original language) = 2'-fluoro modification
  modified_base 6: mod_base = OTHER; note; note (original language) = 2'-O-methyl modification
  modified_base 7..9: mod_base = OTHER; note; note (original language) = 2'-fluoro modification
  modified_base 10..19: mod_base = OTHER; note; note (original language) = 2'-O-methyl modification
  modified_base 1^2: mod_base = OTHER; note; note (original language) = phosphorothioate linkage
  modified_base 2^3: mod_base = OTHER; note; note (original language) = phosphorothioate linkage
aaacggatctccaactaaa

SEQ ID NO: 82 - RNA, 21 nt, synthetic construct
  source 1..21: mol_type = other RNA; note; note (original language) = antisense strand
  modified_base 1: mod_base = OTHER; note; note (original language) = 2'-O-methyl modification
  modified_base 2: mod_base = OTHER; note; note (original language) = 2'-fluoro modification
  modified_base 3..5: mod_base = OTHER; note; note (original language) = 2'-O-methyl modification
  modified_base 6: mod_base = OTHER; note; note (original language) = 2'-fluoro modification
  modified_base 7: mod_base = OTHER; note; note (original language) = 2'-O-methyl modification
  modified_base 8..9: mod_base = OTHER; note; note (original language) = 2'-fluoro modification
  modified_base 10..13: mod_base = OTHER; note; note (original language) = 2'-O-methyl modification
  modified_base 14: mod_base = OTHER; note; note (original language) = 2'-fluoro modification
  modified_base 15: mod_base = OTHER; note; note (original language) = 2'-O-methyl modification
  modified_base 16: mod_base = OTHER; note; note (original language) = 2'-fluoro modification
  modified_base 17..21: mod_base = OTHER; note; note (original language) = 2'-O-methyl modification
  modified_base 1^2: mod_base = OTHER; note; note (original language) = phosphorothioate linkage
  modified_base 2^3: mod_base = OTHER; note; note (original language) = phosphorothioate linkage
  modified_base 19^20: mod_base = OTHER; note; note (original language) = phosphorothioate linkage
  modified_base 20^21: mod_base = OTHER; note; note (original language) = phosphorothioate linkage
tttagttggagatccgtttga

SEQ ID NO: 83 - RNA, 19 nt, synthetic construct
  source 1..19: mol_type = other RNA; note; note (original language) = sense strand
  modified_base 1..6: mod_base = OTHER; note; note (original language) = 2'-O-methyl modification
  modified_base 7..9: mod_base = OTHER; note; note (original language) = 2'-fluoro modification
  modified_base 10..19: mod_base = OTHER; note; note (original language) = 2'-O-methyl modification
  modified_base 1^2: mod_base = OTHER; note; note (original language) = phosphorothioate linkage
  modified_base 2^3: mod_base = OTHER; note; note (original language) = phosphorothioate linkage
aaacggatctccaactaaa

SEQ ID NO: 84 - RNA, 21 nt, synthetic construct
  source 1..21: mol_type = other RNA; note; note (original language) = antisense strand
  modified_base 1: mod_base = OTHER; note; note (original language) = 2'-O-methyl modification
  modified_base 2: mod_base = OTHER; note; note (original language) = 2'-fluoro modification
  modified_base 3..5: mod_base = OTHER; note; note (original language) = 2'-O-methyl modification
  modified_base 6: mod_base = OTHER; note; note (original language) = 2'-fluoro modification
  modified_base 7..13: mod_base = OTHER; note; note (original language) = 2'-O-methyl modification
  modified_base 14: mod_base = OTHER; note; note (original language) = 2'-fluoro modification
  modified_base 15: mod_base = OTHER; note; note (original language) = 2'-O-methyl modification
  modified_base 16: mod_base = OTHER; note; note (original language) = 2'-fluoro modification
  modified_base 17..21: mod_base = OTHER; note; note (original language) = 2'-O-methyl modification
  modified_base 1^2: mod_base = OTHER; note; note (original language) = phosphorothioate linkage
  modified_base 2^3: mod_base = OTHER; note; note (original language) = phosphorothioate linkage
  modified_base 19^20: mod_base = OTHER; note; note (original language) = phosphorothioate linkage
  modified_base 20^21: mod_base = OTHER; note; note (original language) = phosphorothioate linkage
tttagttggagatccgtttga